European Patent Application EP 4 389 768 A1, published June 26, 2024. Title: ANTI-B7-H4 ANTIBODY, AND PREPARATION METHOD THEREFOR AND USE THEREOF. Applicant: Harbour Biomed (Shanghai) Co., Ltd. The sequence listing filed with the application follows.

SEQUENCE LISTING (88 sequences)

SEQ ID NO: 1 - protein, 25 aa, synthetic construct
EVQLVESGGGLVQPGGSLKLSCAAS

SEQ ID NO: 2 - protein, 25 aa, synthetic construct [sequence omitted]

SEQ ID NO: 3 - protein, 7 aa, synthetic construct
GFTFSTY

SEQ ID NO: 4 - protein, 7 aa, synthetic construct
GFAFSNY

SEQ ID NO: 5 - protein, 7 aa, synthetic construct
GFTFTDF

SEQ ID NO: 6 - protein, 19 aa, synthetic construct
AMNWVRQASGKGLEWVGRI

SEQ ID NO: 7 - protein, 19 aa, synthetic construct
WMHWARQVPGKGRVWISRI

SEQ ID NO: 8 - protein, 19 aa, synthetic construct
WMHWVRQVPGKGREWVSRI

SEQ ID NO: 9 - protein, 19 aa, synthetic construct
WMHWARQVPGKGREWISRI

SEQ ID NO: 10 - protein, 8 aa, synthetic construct
RSKYNNYA

SEQ ID NO: 11 - protein, 6 aa, synthetic construct
SGDGRS

SEQ ID NO: 12 - protein, 6 aa, synthetic construct
SPDGSS

SEQ ID NO: 13 - protein, 6 aa, synthetic construct
SGDSDS

SEQ ID NO: 14 - protein, 6 aa, synthetic construct
SGDSES

SEQ ID NO: 15 - protein, 6 aa, synthetic construct
SGDSSS

SEQ ID NO: 16 - protein, 6 aa, synthetic construct
SGDSTS

SEQ ID NO: 17 - protein, 6 aa, synthetic construct
SGDSRS

SEQ ID NO: 18 - protein, 6 aa, synthetic construct
SPDSSS

SEQ ID NO: 19 - protein, 41 aa, synthetic construct
TYYADSVKDRFTISRDDSKNTAYLQMNSLKTEDTAVYYCTR

SEQ ID NO: 20 - protein, 41 aa, synthetic construct
TSYADSVKGRFTISRDNAKNMVYLQMNNLRAEDTAVYYCAR

SEQ ID NO: 21 - protein, 41 aa, synthetic construct
TSYEDSVKGRFTISRDNAKNTVYLQMHGLRAEDTAVYYCTR

SEQ ID NO: 22 - protein, 41 aa, synthetic construct
TSYEDSVKGRFTISRDNAKNMVYLQMNNLRAEDTAVYYCAR

SEQ ID NO: 23 - protein, 14 aa, synthetic construct
HGNFGNSYVSWFAY

SEQ ID NO: 24 - protein, 13 aa, synthetic construct
DRFGDDYYYGMNV

SEQ ID NO: 25 - protein, 13 aa, synthetic construct
FSTGWHRIEYFQH

SEQ ID NO: 26 - protein, 11 aa, synthetic construct
WGQGTLVTVSS

SEQ ID NO: 27 - protein, 11 aa, synthetic construct
WGQGTTVTVSS

SEQ ID NO: 28 - protein, 22 aa, synthetic construct
QAVVTQEPSLTVSPGGTVTLTC

SEQ ID NO: 29 - protein, 14 aa, synthetic construct
RSSTGAVTTSNYAN

SEQ ID NO: 30 - protein, 15 aa, synthetic construct
WVQQKPGQAPRGLIG

SEQ ID NO: 31 - protein, 7 aa, synthetic construct
GTNKRAP

SEQ ID NO: 32 - protein, 32 aa, synthetic construct
WTPARFSGSLLGDKAALTLLGAQPEDEAEYFC

SEQ ID NO: 33 - protein, 9 aa, synthetic construct
ALWYSNLWV

SEQ ID NO: 34 - protein, 10 aa, synthetic construct
FGGGTKLTVL

SEQ ID NO: 35 - protein, 125 aa, synthetic construct
EVQLVESGGGLVQPGGSLKLSCAASGFTFSTYAMNWVRQASGKGLEWVGRIRSKYNNYATYYADSVKDRFTISRDDSKNTAYLQMNSLKTEDTAVYYCTRHGNFGNSYVSWFAYWGQGTLVTVSS

SEQ ID NO: 36 - protein, 122 aa, synthetic construct
EVQLVESGGGLVQPGGSLRLSCAASGFAFSNYWMHWARQVPGKGRVWISRISGDGRSTSYADSVKGRFTISRDNAKNMVYLQMNNLRAEDTAVYYCARDRFGDDYYYGMNVWGQGTTVTVSS

SEQ ID NO: 37 - protein, 122 aa, synthetic construct
EVQLVESGGGLVQPGGSLRLSCAASGFTFTDFWMHWVRQVPGKGREWVSRISPDGSSTSYEDSVKGRFTISRDNAKNTVYLQMHGLRAEDTAVYYCTRFSTGWHRIEYFQHWGQGTLVTVSS

SEQ ID NO: 38 - protein, 122 aa, synthetic construct
EVQLVESGGGLVQPGGSLRLSCAASGFAFSNYWMHWARQVPGKGREWISRISGDSDSTSYEDSVKGRFTISRDNAKNMVYLQMNNLRAEDTAVYYCARDRFGDDYYYGMNVWGQGTTVTVSS

SEQ ID NO: 39 - protein, 122 aa, synthetic construct
EVQLVESGGGLVQPGGSLRLSCAASGFAFSNYWMHWARQVPGKGREWISRISGDSESTSYADSVKGRFTISRDNAKNMVYLQMNNLRAEDTAVYYCARDRFGDDYYYGMNVWGQGTTVTVSS

SEQ ID NO: 40 - protein, 122 aa, synthetic construct
EVQLVESGGGLVQPGGSLRLSCAASGFAFSNYWMHWARQVPGKGREWISRISGDSSSTSYADSVKGRFTISRDNAKNMVYLQMNNLRAEDTAVYYCARDRFGDDYYYGMNVWGQGTTVTVSS

SEQ ID NO: 41 - protein, 122 aa, synthetic construct
EVQLVESGGGLVQPGGSLRLSCAASGFAFSNYWMHWARQVPGKGREWISRISGDSSSTSYEDSVKGRFTISRDNAKNMVYLQMNNLRAEDTAVYYCARDRFGDDYYYGMNVWGQGTTVTVSS

SEQ ID NO: 42 - protein, 122 aa, synthetic construct
EVQLVESGGGLVQPGGSLRLSCAASGFAFSNYWMHWARQVPGKGREWISRISGDSTSTSYADSVKGRFTISRDNAKNMVYLQMNNLRAEDTAVYYCARDRFGDDYYYGMNVWGQGTTVTVSS

SEQ ID NO: 43 - protein, 122 aa, synthetic construct
EVQLVESGGGLVQPGGSLRLSCAASGFAFSNYWMHWARQVPGKGREWISRISGDSTSTSYEDSVKGRFTISRDNAKNMVYLQMNNLRAEDTAVYYCARDRFGDDYYYGMNVWGQGTTVTVSS

SEQ ID NO: 44 - protein, 122 aa, synthetic construct
EVQLVESGGGLVQPGGSLRLSCAASGFAFSNYWMHWARQVPGKGRVWISRISGDSRSTSYADSVKGRFTISRDNAKNMVYLQMNNLRAEDTAVYYCARDRFGDDYYYGMNVWGQGTTVTVSS

SEQ ID NO: 45 - protein, 122 aa, synthetic construct
EVQLVESGGGLVQPGGSLRLSCAASGFTFTDFWMHWVRQVPGKGREWVSRISPDSSSTSYEDSVKGRFTISRDNAKNTVYLQMHGLRAEDTAVYYCTRFSTGWHRIEYFQHWGQGTLVTVSS

SEQ ID NO: 46 - protein, 109 aa, synthetic construct
QAVVTQEPSLTVSPGGTVTLTCRSSTGAVTTSNYANWVQQKPGQAPRGLIGGTNKRAPWTPARFSGSLLGDKAALTLLGAQPEDEAEYFCALWYSNLWVFGGGTKLTVL

SEQ ID NO: 47 - protein, 455 aa, synthetic construct
EVQLVESGGGLVQPGGSLKLSCAASGFTFSTYAMNWVRQASGKGLEWVGRIRSKYNNYATYYADSVKDRFTISRDDSKNTAYLQMNSLKTEDTAVYYCTRHGNFGNSYVSWFAYWGQGTLVTVSSASTKGPSVFPLAPSSKSTSGGTAALGCLVKDYFPEPVTVSWNSGALTSGVHTFPAVLQSSGLYSLSSVVTVPSSSLGTQTYICNVNHKPSNTKVDKKVEPKSCDKTHTCPPCPAPEAAGGPSVFLFPPKPKDTLMISRTPEVTCVVVDVSHEDPEVKFNWYVDGVEVHNAKTKPREEQYNSTYRVVSVLTVLHQDWLNGKEYKCKVSNKALPAPIEKTISKAKGQPREPQVYTLPPSREEMTKNQVSLTCLVKGFYPSDIAVEWESNGQPENNYKTTPPVLDSDGSFFLYSKLTVDKSRWQQGNVFSCSVMHEALHNHYTQKSLSLSPGK

SEQ ID NO: 48 - protein, 354 aa, synthetic construct
EVQLVESGGGLVQPGGSLRLSCAASGFAFSNYWMHWARQVPGKGRVWISRISGDGRSTSYADSVKGRFTISRDNAKNMVYLQMNNLRAEDTAVYYCARDRFGDDYYYGMNVWGQGTTVTVSSEPKSSDKTHTCPPCPAPELLGGPSVFLFPPKPKDTLMISRTPEVTCVVVDVSHEDPEVKFNWYVDGVEVHNAKTKPREEQYNSTYRVVSVLTVLHQDWLNGKEYKCKVSNKALPAPIEKTISKAKGQPREPQVYTLPPSREEMTKNQVSLTCLVKGFYPSDIAVEWESNGQPENNYKTTPPVLDSDGSFFLYSKLTVDKSRWQQGNVFSCSVMHEALHNHYTQKSLSLSPGK

SEQ ID NO: 49 - protein, 354 aa, synthetic construct
EVQLVESGGGLVQPGGSLRLSCAASGFTFTDFWMHWVRQVPGKGREWVSRISPDGSSTSYEDSVKGRFTISRDNAKNTVYLQMHGLRAEDTAVYYCTRFSTGWHRIEYFQHWGQGTLVTVSSEPKSSDKTHTCPPCPAPELLGGPSVFLFPPKPKDTLMISRTPEVTCVVVDVSHEDPEVKFNWYVDGVEVHNAKTKPREEQYNSTYRVVSVLTVLHQDWLNGKEYKCKVSNKALPAPIEKTISKAKGQPREPQVYTLPPSREEMTKNQVSLTCLVKGFYPSDIAVEWESNGQPENNYKTTPPVLDSDGSFFLYSKLTVDKSRWQQGNVFSCSVMHEALHNHYTQKSLSLSPGK

SEQ ID NO: 50 - protein, 354 aa, synthetic construct
EVQLVESGGGLVQPGGSLRLSCAASGFAFSNYWMHWARQVPGKGREWISRISGDSDSTSYEDSVKGRFTISRDNAKNMVYLQMNNLRAEDTAVYYCARDRFGDDYYYGMNVWGQGTTVTVSSEPKSSDKTHTCPPCPAPELLGGPSVFLFPPKPKDTLMISRTPEVTCVVVDVSHEDPEVKFNWYVDGVEVHNAKTKPREEQYNSTYRVVSVLTVLHQDWLNGKEYKCKVSNKALPAPIEKTISKAKGQPREPQVYTLPPSREEMTKNQVSLTCLVKGFYPSDIAVEWESNGQPENNYKTTPPVLDSDGSFFLYSKLTVDKSRWQQGNVFSCSVMHEALHNHYTQKSLSLSPGK

SEQ ID NO: 51 - protein, 354 aa, synthetic construct
EVQLVESGGGLVQPGGSLRLSCAASGFAFSNYWMHWARQVPGKGREWISRISGDSESTSYADSVKGRFTISRDNAKNMVYLQMNNLRAEDTAVYYCARDRFGDDYYYGMNVWGQGTTVTVSSEPKSSDKTHTCPPCPAPELLGGPSVFLFPPKPKDTLMISRTPEVTCVVVDVSHEDPEVKFNWYVDGVEVHNAKTKPREEQYNSTYRVVSVLTVLHQDWLNGKEYKCKVSNKALPAPIEKTISKAKGQPREPQVYTLPPSREEMTKNQVSLTCLVKGFYPSDIAVEWESNGQPENNYKTTPPVLDSDGSFFLYSKLTVDKSRWQQGNVFSCSVMHEALHNHYTQKSLSLSPGK

SEQ ID NO: 52 - protein, 354 aa, synthetic construct
EVQLVESGGGLVQPGGSLRLSCAASGFAFSNYWMHWARQVPGKGREWISRISGDSSSTSYADSVKGRFTISRDNAKNMVYLQMNNLRAEDTAVYYCARDRFGDDYYYGMNVWGQGTTVTVSSEPKSSDKTHTCPPCPAPELLGGPSVFLFPPKPKDTLMISRTPEVTCVVVDVSHEDPEVKFNWYVDGVEVHNAKTKPREEQYNSTYRVVSVLTVLHQDWLNGKEYKCKVSNKALPAPIEKTISKAKGQPREPQVYTLPPSREEMTKNQVSLTCLVKGFYPSDIAVEWESNGQPENNYKTTPPVLDSDGSFFLYSKLTVDKSRWQQGNVFSCSVMHEALHNHYTQKSLSLSPGK

SEQ ID NO: 53 - protein, 354 aa, synthetic construct
EVQLVESGGGLVQPGGSLRLSCAASGFAFSNYWMHWARQVPGKGREWISRISGDSSSTSYEDSVKGRFTISRDNAKNMVYLQMNNLRAEDTAVYYCARDRFGDDYYYGMNVWGQGTTVTVSSEPKSSDKTHTCPPCPAPELLGGPSVFLFPPKPKDTLMISRTPEVTCVVVDVSHEDPEVKFNWYVDGVEVHNAKTKPREEQYNSTYRVVSVLTVLHQDWLNGKEYKCKVSNKALPAPIEKTISKAKGQPREPQVYTLPPSREEMTKNQVSLTCLVKGFYPSDIAVEWESNGQPENNYKTTPPVLDSDGSFFLYSKLTVDKSRWQQGNVFSCSVMHEALHNHYTQKSLSLSPGK

SEQ ID NO: 54 - protein, 354 aa, synthetic construct
EVQLVESGGGLVQPGGSLRLSCAASGFAFSNYWMHWARQVPGKGREWISRISGDSTSTSYADSVKGRFTISRDNAKNMVYLQMNNLRAEDTAVYYCARDRFGDDYYYGMNVWGQGTTVTVSSEPKSSDKTHTCPPCPAPELLGGPSVFLFPPKPKDTLMISRTPEVTCVVVDVSHEDPEVKFNWYVDGVEVHNAKTKPREEQYNSTYRVVSVLTVLHQDWLNGKEYKCKVSNKALPAPIEKTISKAKGQPREPQVYTLPPSREEMTKNQVSLTCLVKGFYPSDIAVEWESNGQPENNYKTTPPVLDSDGSFFLYSKLTVDKSRWQQGNVFSCSVMHEALHNHYTQKSLSLSPGK

SEQ ID NO: 55 - protein, 354 aa, synthetic construct
EVQLVESGGGLVQPGGSLRLSCAASGFAFSNYWMHWARQVPGKGREWISRISGDSTSTSYEDSVKGRFTISRDNAKNMVYLQMNNLRAEDTAVYYCARDRFGDDYYYGMNVWGQGTTVTVSSEPKSSDKTHTCPPCPAPELLGGPSVFLFPPKPKDTLMISRTPEVTCVVVDVSHEDPEVKFNWYVDGVEVHNAKTKPREEQYNSTYRVVSVLTVLHQDWLNGKEYKCKVSNKALPAPIEKTISKAKGQPREPQVYTLPPSREEMTKNQVSLTCLVKGFYPSDIAVEWESNGQPENNYKTTPPVLDSDGSFFLYSKLTVDKSRWQQGNVFSCSVMHEALHNHYTQKSLSLSPGK

SEQ ID NO: 56 - protein, 354 aa, synthetic construct
EVQLVESGGGLVQPGGSLRLSCAASGFAFSNYWMHWARQVPGKGRVWISRISGDSRSTSYADSVKGRFTISRDNAKNMVYLQMNNLRAEDTAVYYCARDRFGDDYYYGMNVWGQGTTVTVSSEPKSSDKTHTCPPCPAPELLGGPSVFLFPPKPKDTLMISRTPEVTCVVVDVSHEDPEVKFNWYVDGVEVHNAKTKPREEQYNSTYRVVSVLTVLHQDWLNGKEYKCKVSNKALPAPIEKTISKAKGQPREPQVYTLPPSREEMTKNQVSLTCLVKGFYPSDIAVEWESNGQPENNYKTTPPVLDSDGSFFLYSKLTVDKSRWQQGNVFSCSVMHEALHNHYTQKSLSLSPGK

SEQ ID NO: 57 - protein, 354 aa, synthetic construct
EVQLVESGGGLVQPGGSLRLSCAASGFTFTDFWMHWVRQVPGKGREWVSRISPDSSSTSYEDSVKGRFTISRDNAKNTVYLQMHGLRAEDTAVYYCTRFSTGWHRIEYFQHWGQGTLVTVSSEPKSSDKTHTCPPCPAPELLGGPSVFLFPPKPKDTLMISRTPEVTCVVVDVSHEDPEVKFNWYVDGVEVHNAKTKPREEQYNSTYRVVSVLTVLHQDWLNGKEYKCKVSNKALPAPIEKTISKAKGQPREPQVYTLPPSREEMTKNQVSLTCLVKGFYPSDIAVEWESNGQPENNYKTTPPVLDSDGSFFLYSKLTVDKSRWQQGNVFSCSVMHEALHNHYTQKSLSLSPGK

SEQ ID NO: 58 - protein, 215 aa, synthetic construct
QAVVTQEPSLTVSPGGTVTLTCRSSTGAVTTSNYANWVQQKPGQAPRGLIGGTNKRAPWTPARFSGSLLGDKAALTLLGAQPEDEAEYFCALWYSNLWVFGGGTKLTVLGQPKAAPSVTLFPPSSEELQANKATLVCLISDFYPGAVTVAWKADSSPVKAGVETTTPSKQSNNKYAASSYLSLTPEQWKSHRSYSCQVTHEGSTVEKTVAPTECS

SEQ ID NO: 59 - protein, 455 aa, synthetic construct
EVQLVESGGGLVQPGGSLKLSCAASGFTFSTYAMNWVRQASGKGLEWVGRIRSKYNNYATYYADSVKDRFTISRDDSKNTAYLQMNSLKTEDTAVYYCTRHGNFGNSYVSWFAYWGQGTLVTVSSASTKGPSVFPLAPSSKSTSGGTAALGCLVKDYFPEPVTVSWNSGALTSGVHTFPAVLQSSGLYSLSSVVTVPSSSLGTQTYICNVNHKPSNTKVDKKVEPKSCDKTHTCPPCPAPEAAGAPSVFLFPPKPKDTLMISRTPEVTCVVVDVSHEDPEVKFNWYVDGVEVHNAKTKPREEQYNSTYRVVSVLTVLHQDWLNGKEYKCKVSNKALPAPIEKTISKAKGQPREPQVYTLPPCREEMTKNQVSLWCLVKGFYPSDIAVEWESNGQPENNYKTTPPVLDSDGSFFLYSKLTVDKSRWQQGNVFSCSVMHEALHNHYTQKSLSLSPGK

SEQ ID NO: 60 - protein, 493 aa, synthetic construct
EVQLVESGGGLVQPGGSLRLSCAASGFAFSNYWMHWARQVPGKGRVWISRISGDSRSTSYADSVKGRFTISRDNAKNMVYLQMNNLRAEDTAVYYCARDRFGDDYYYGMNVWGQGTTVTVSSGGGGSGGGGSGGGGSEVQLVESGGGLVQPGGSLRLSCAASGFAFSNYWMHWARQVPGKGRVWISRISGDSRSTSYADSVKGRFTISRDNAKNMVYLQMNNLRAEDTAVYYCARDRFGDDYYYGMNVWGQGTTVTVSSASEPKSSDKTHTCPPCPAPEAAGAPSVFLFPPKPKDTLMISRTPEVTCVVVDVSHEDPEVKFNWYVDGVEVHNAKTKPREEQYNSTYRVVSVLTVLHQDWLNGKEYKCKVSNKALPAPIEKTISKAKGQPREPQVCTLPPSREEMTKNQVSLSCAVKGFYPSDIAVEWESNGQPENNYKTTPPVLDSDGSFFLVSKLTVDKSRWQQGNVFSCSVMHEALHNHYTQKSLSLSPGK

SEQ ID NO: 61 - protein, 493 aa, synthetic construct
EVQLVESGGGLVQPGGSLRLSCAASGFTFTDFWMHWVRQVPGKGREWVSRISPDSSSTSYEDSVKGRFTISRDNAKNTVYLQMHGLRAEDTAVYYCTRFSTGWHRIEYFQHWGQGTLVTVSSGGGGSGGGGSGGGGSEVQLVESGGGLVQPGGSLRLSCAASGFTFTDFWMHWVRQVPGKGREWVSRISPDSSSTSYEDSVKGRFTISRDNAKNTVYLQMHGLRAEDTAVYYCTRFSTGWHRIEYFQHWGQGTLVTVSSASEPKSSDKTHTCPPCPAPEAAGAPSVFLFPPKPKDTLMISRTPEVTCVVVDVSHEDPEVKFNWYVDGVEVHNAKTKPREEQYNSTYRVVSVLTVLHQDWLNGKEYKCKVSNKALPAPIEKTISKAKGQPREPQVCTLPPSREEMTKNQVSLSCAVKGFYPSDIAVEWESNGQPENNYKTTPPVLDSDGSFFLVSKLTVDKSRWQQGNVFSCSVMHEALHNHYTQKSLSLSPGK

SEQ ID NO: 62 - protein, 493 aa, synthetic construct
EVQLVESGGGLVQPGGSLRLSCAASGFAFSNYWMHWARQVPGKGRVWISRISGDSRSTSYADSVKGRFTISRDNAKNMVYLQMNNLRAEDTAVYYCARDRFGDDYYYGMNVWGQGTTVTVSSGGGGSGGGGSGGGGSEVQLVESGGGLVQPGGSLRLSCAASGFTFTDFWMHWVRQVPGKGREWVSRISPDSSSTSYEDSVKGRFTISRDNAKNTVYLQMHGLRAEDTAVYYCTRFSTGWHRIEYFQHWGQGTLVTVSSASEPKSSDKTHTCPPCPAPEAAGAPSVFLFPPKPKDTLMISRTPEVTCVVVDVSHEDPEVKFNWYVDGVEVHNAKTKPREEQYNSTYRVVSVLTVLHQDWLNGKEYKCKVSNKALPAPIEKTISKAKGQPREPQVCTLPPSREEMTKNQVSLSCAVKGFYPSDIAVEWESNGQPENNYKTTPPVLDSDGSFFLVSKLTVDKSRWQQGNVFSCSVMHEALHNHYTQKSLSLSPGK

SEQ ID NO: 63 - protein, 493 aa, synthetic construct
EVQLVESGGGLVQPGGSLRLSCAASGFAFSNYWMHWARQVPGKGRVWICRISGDSRSTSYADSVKGRFTCSRDNAKNMVYLQMNNLRAEDTAVYYCARDRFGDDYYYGMNVWGQGTTVTVSSGGGGSGGGGSGGGGSEVQLVESGGGLVQPGGSLRLSCAASGFAFSNYWMHWARQVPGKGRVWICRISGDSRSTSYADSVKGRFTCSRDNAKNMVYLQMNNLRAEDTAVYYCARDRFGDDYYYGMNVWGQGTTVTVSSASEPKSSDKTHTCPPCPAPEAAGAPSVFLFPPKPKDTLMISRTPEVTCVVVDVSHEDPEVKFNWYVDGVEVHNAKTKPREEQYNSTYRVVSVLTVLHQDWLNGKEYKCKVSNKALPAPIEKTISKAKGQPREPQVCTLPPSREEMTKNQVSLSCAVKGFYPSDIAVEWESNGQPENNYKTTPPVLDSDGSFFLVSKLTVDKSRWQQGNVFSCSVMHEALHNHYTQKSLSLSPGK

SEQ ID NO: 64 - protein, 493 aa, synthetic construct
EVQLVESGGGLVQPGGSLRLSCAASGFTFTDFWMHWVRQVPGKGREWVCRISPDSSSTSYEDSVKGRFTCSRDNAKNTVYLQMHGLRAEDTAVYYCTRFSTGWHRIEYFQHWGQGTLVTVSSGGGGSGGGGSGGGGSEVQLVESGGGLVQPGGSLRLSCAASGFTFTDFWMHWVRQVPGKGREWVCRISPDSSSTSYEDSVKGRFTCSRDNAKNTVYLQMHGLRAEDTAVYYCTRFSTGWHRIEYFQHWGQGTLVTVSSASEPKSSDKTHTCPPCPAPEAAGAPSVFLFPPKPKDTLMISRTPEVTCVVVDVSHEDPEVKFNWYVDGVEVHNAKTKPREEQYNSTYRVVSVLTVLHQDWLNGKEYKCKVSNKALPAPIEKTISKAKGQPREPQVCTLPPSREEMTKNQVSLSCAVKGFYPSDIAVEWESNGQPENNYKTTPPVLDSDGSFFLVSKLTVDKSRWQQGNVFSCSVMHEALHNHYTQKSLSLSPGK

SEQ ID NO: 65 - protein, 493 aa, synthetic construct
EVQLVESGGGLVQPGGSLRLSCAASGFAFSNYWMHWARQVPGKGRVWICRISGDSRSTSYADSVKGRFTCSRDNAKNMVYLQMNNLRAEDTAVYYCARDRFGDDYYYGMNVWGQGTTVTVSSGGGGSGGGGSGGGGSEVQLVESGGGLVQPGGSLRLSCAASGFTFTDFWMHWVRQVPGKGREWVCRISPDSSSTSYEDSVKGRFTCSRDNAKNTVYLQMHGLRAEDTAVYYCTRFSTGWHRIEYFQHWGQGTLVTVSSASEPKSSDKTHTCPPCPAPEAAGAPSVFLFPPKPKDTLMISRTPEVTCVVVDVSHEDPEVKFNWYVDGVEVHNAKTKPREEQYNSTYRVVSVLTVLHQDWLNGKEYKCKVSNKALPAPIEKTISKAKGQPREPQVCTLPPSREEMTKNQVSLSCAVKGFYPSDIAVEWESNGQPENNYKTTPPVLDSDGSFFLVSKLTVDKSRWQQGNVFSCSVMHEALHNHYTQKSLSLSPGK

SEQ ID NO: 66 - protein, 15 aa, synthetic construct
GGGGSGGGGSGGGGS

SEQ ID NO: 67 - protein, 217 aa, synthetic construct
APEAAGAPSVFLFPPKPKDTLMISRTPEVTCVVVDVSHEDPEVKFNWYVDGVEVHNAKTKPREEQYNSTYRVVSVLTVLHQDWLNGKEYKCKVSNKALPAPIEKTISKAKGQPREPQVCTLPPSREEMTKNQVSLSCAVKGFYPSDIAVEWESNGQPENNYKTTPPVLDSDGSFFLVSKLTVDKSRWQQGNVFSCSVMHEALHNHYTQKSLSLSPGK

SEQ ID NO: 68 - protein, 217 aa, synthetic construct
APEAAGAPSVFLFPPKPKDTLMISRTPEVTCVVVDVSHEDPEVKFNWYVDGVEVHNAKTKPREEQYNSTYRVVSVLTVLHQDWLNGKEYKCKVSNKALPAPIEKTISKAKGQPREPQVYTLPPCREEMTKNQVSLWCLVKGFYPSDIAVEWESNGQPENNYKTTPPVLDSDGSFFLYSKLTVDKSRWQQGNVFSCSVMHEALHNHYTQKSLSLSPGK

SEQ ID NO: 69 - protein, 356 aa, synthetic construct
EVQLVESGGGLVQPGGSLRLSCAASGFAFSNYWMHWARQVPGKGRVWICRISGDSRSTSYADSVKGRFTCSRDNAKNMVYLQMNNLRAEDTAVYYCARDRFGDDYYYGMNVWGQGTTVTVSSASEPKSSDKTHTCPPCPAPEAAGAPSVFLFPPKPKDTLMISRTPEVTCVVVDVSHEDPEVKFNWYVDGVEVHNAKTKPREEQYNSTYRVVSVLTVLHQDWLNGKEYKCKVSNKALPAPIEKTISKAKGQPREPQVCTLPPSREEMTKNQVSLSCAVKGFYPSDIAVEWESNGQPENNYKTTPPVLDSDGSFFLVSKLTVDKSRWQQGNVFSCSVMHEALHNHYTQKSLSLSPGK

SEQ ID NO: 70 - protein, 356 aa, synthetic construct
EVQLVESGGGLVQPGGSLRLSCAASGFTFTDFWMHWVRQVPGKGREWVCRISPDSSSTSYEDSVKGRFTCSRDNAKNTVYLQMHGLRAEDTAVYYCTRFSTGWHRIEYFQHWGQGTLVTVSSASEPKSSDKTHTCPPCPAPEAAGAPSVFLFPPKPKDTLMISRTPEVTCVVVDVSHEDPEVKFNWYVDGVEVHNAKTKPREEQYNSTYRVVSVLTVLHQDWLNGKEYKCKVSNKALPAPIEKTISKAKGQPREPQVCTLPPSREEMTKNQVSLSCAVKGFYPSDIAVEWESNGQPENNYKTTPPVLDSDGSFFLVSKLTVDKSRWQQGNVFSCSVMHEALHNHYTQKSLSLSPGK

SEQ ID NO: 71 - protein, 25 aa, synthetic construct
QVQLVQSGAEVKKPGSSMRVSCKAS

SEQ ID NO: 72 - protein, 7 aa, synthetic construct
EDTFSSY

SEQ ID NO: 73 - protein, 19 aa, synthetic construct
AISWVRQAPGQGLEWMGGT

SEQ ID NO: 74 - protein, 6 aa, synthetic construct
APIFGT

SEQ ID NO: 75 - protein, 41 aa, synthetic construct
TNYAQKFQGRVTITADKSTSTAYMELSSLRSEDTAVYYCAR

SEQ ID NO: 76 - protein, 7 aa, synthetic construct
GGPYFDY

SEQ ID NO: 77 - protein, 23 aa, synthetic construct
EIVMTQSPASLSVSPGERATLSC

SEQ ID NO: 78 - protein, 11 aa, synthetic construct
RASQSVSSNLA

SEQ ID NO: 79 - protein, 15 aa, synthetic construct
WYQQKPGQAPRLLIY

SEQ ID NO: 80 - protein, 7 aa, synthetic construct
GASTRAT

SEQ ID NO: 81 - protein, 32 aa, synthetic construct
GIPARVSGGGSGTEFTLTISSLQSEDFAVYYC

SEQ ID NO: 82 - protein, 9 aa, synthetic construct
QQYKNWPFT

SEQ ID NO: 83 - protein, 10 aa, synthetic construct
FGPGTKLEIK

SEQ ID NO: 84 - protein, 116 aa, synthetic construct
QVQLVQSGAEVKKPGSSMRVSCKASEDTFSSYAISWVRQAPGQGLEWMGGTAPIFGTTNYAQKFQGRVTITADKSTSTAYMELSSLRSEDTAVYYCARGGPYFDYWGQGTLVTVSS

SEQ ID NO: 85 - protein, 107 aa, synthetic construct
EIVMTQSPASLSVSPGERATLSCRASQSVSSNLAWYQQKPGQAPRLLIYGASTRATGIPARVSGGGSGTEFTLTISSLQSEDFAVYYCQQYKNWPFTFGPGTKLEIK

SEQ ID NO: 86 - protein, 477 aa, synthetic construct
EIVMTQSPASLSVSPGERATLSCRASQSVSSNLAWYQQKPGQAPRLLIYGASTRATGIPARVSGGGSGTEFTLTISSLQSEDFAVYYCQQYKNWPFTFGPGTKLEIKGGGGSGGGGSGGGGSGGGGSQVQLVQSGAEVKKPGSSMRVSCKASEDTFSSYAISWVRQAPGQGLEWMGGTAPIFGTTNYAQKFQGRVTITADKSTSTAYMELSSLRSEDTAVYYCARGGPYFDYWGQGTLVTVSSASEPKSSDKTHTCPPCPAPEAAGAPSVFLFPPKPKDTLMISRTPEVTCVVVDVSHEDPEVKFNWYVDGVEVHNAKTKPREEQYNSTYRVVSVLTVLHQDWLNGKEYKCKVSNKALPAPIEKTISKAKGQPREPQVCTLPPSREEMTKNQVSLSCAVKGFYPSDIAVEWESNGQPENNYKTTPPVLDSDGSFFLVSKLTVDKSRWQQGNVFSCSVMHEALHNHYTQKSLSLSPGK

SEQ ID NO: 87 - protein, 480 aa, synthetic construct
EIVMTQSPASLSVSPGERATLSCRASQSVSSNLAWYQQKPGQAPRLLIYGASTRATGIPARVSGGGSGTEFTLTISSLQSEDFAVYYCQQYKNWPFTFGPGTKLEIKGGGGSGGGGSGGGGSGGGGSQVQLVQSGAEVKKPGSSMRVSCKASEDTFSSYAISWVRQAPGQGLEWMGGTAPIFGTTNYAQKFQGRVTITADKSTSTAYMELSSLRSEDTAVYYCARGGPYFDYWGQGTLVTVSSGGGASEPKSCDKTHTCPPCPAPELLGGPSVFLFPPKPKDTLMISRTPEVTCVVVDVSHEDPEVKFNWYVDGVEVHNAKTKPREEQYNSTYRVVSVLTVLHQDWLNGKEYKCKVSNKALPAPIEKTISKAKGQPREPQVYTLPPSREEMTKNQVSLTCLVKGFYPSDIAVEWESNGQPENNYKTTPPVLDSDGSFFLYSKLTVDKSRWQQGNVFSCSVMHEALHNHYTQKSLSLSPGK

SEQ ID NO: 88 - protein, 20 aa, synthetic construct
GGGGSGGGGSGGGGSGGGGS